European Patent Specification EP 3 877 396 B1, published February 19, 2025. Title: Polypeptides for the Treatment of Stress, Immunoreaction and Stroke Syndromes. Applicant: Neopep Pharma GmbH & Co. KG. The sequence listing filed with the application follows.

SEQUENCE LISTING (15 sequences)

SEQ ID NO: 1 - protein, 12 aa, human
LVRYTQKAPQVS

SEQ ID NO: 2 - protein, 12 aa, human
MVRYTQKAPQVS

SEQ ID NO: 3 - protein, 12 aa, human
VVRYTQKAPQVS

SEQ ID NO: 4 - protein, 12 aa, human
LMRYTQKQPQVS

SEQ ID NO: 5 - protein, 12 aa, human
LLRYTQKQPQVS

SEQ ID NO: 6 - protein, 12 aa, human
LVKYTQKQPQVS

SEQ ID NO: 7 - protein, 12 aa, human
LVCYTQKQPQVS

SEQ ID NO: 8 - protein, 12 aa, human
LVRWTQKAPQVS

SEQ ID NO: 9 - protein, 12 aa, human
LVRYSQKQPQVS

SEQ ID NO: 10 - protein, 12 aa, human
LVRYTCKAPQVS

SEQ ID NO: 11 - protein, 12 aa, human
LVRYTQCAPQVS

SEQ ID NO: 12 - protein, 12 aa, human
LVRYTQRAPQVS

SEQ ID NO: 13 - protein, 12 aa, human
LVRYTQKAPCVS

SEQ ID NO: 14 - protein, 12 aa, human
LVRYTQKAPQMS

SEQ ID NO: 15 - protein, 12 aa, human
LVRYTQKAPQFS